European Patent Application EP 4 261 284 A1, published October 18, 2023. Title: Stable target editing guide RNA with chemically modified nucleic acid. Applicant: FUKUOKA UNIVERSITY DAIICHI SANKYO COMPANY, LIMITED. The sequence listing filed with the application follows.

SEQUENCE LISTING (112 sequences)

SEQ ID NO: 1 - RNA, 24 nt, Artificial Sequence
  gRNA
cagcucaaccaagcggugagguac

SEQ ID NO: 2 - RNA, 25 nt, Artificial Sequence
  target
guaccucaccgcuuaguucgagcug

SEQ ID NO: 3 - RNA, 200 nt, Artificial Sequence
  Target hGAPDH
gggccucuucgcuauuacgccagcuggcgaaagggggaugugcugcaaggcgauuaaguuggguaacgccaggguuuucccagucacgacguuguaaaacgacggccagugaauucucuccccuccucacaguugccauguagaccccuugaagaggggaggggccuaagcuuggcguaaucauggucauagcuguuucc

SEQ ID NO: 4 - RNA, 24 nt, Artificial Sequence
  gRNA
ucaaggguccacauggcaacugug

SEQ ID NO: 5 - RNA, 910 nt, Artificial Sequence
  Target Rluc WT
accauggcuuccaagguguacgaccccgagcaacgcaaacgcaugaucacugggccucaguggugggcucgcugcaagcaaaugaacgugcuggacuccuucaucaacuacuaugauuccgagaagcacgccgagaacgccgugauuuuucugcaugguaacgcugccuccagcuaccuguggaggcacgucgugccucacaucgagcccguggcuagaugcaucaucccugaucugaucggaauggguaaguccggcaagagcgggaauggcucauaucgccuccuggaucacuacaaguaccucaccgcuugguucgagcugcugaaccuuccaaagaaaaucaucuuugugggccacgacuggggggcuugucuggccuuucacuacuccuacgagcaccaagacaagaucaaggccaucguccaugcugagagugucguggacgugaucgaguccugggacgaguggccugacaucgaggaggauaucgcccugaucaagagcgaagagggcgagaaaauggugcuugagaauaacuucuucgucgagaccaugcucccaagcaagaucaugcggaaacuggagccugaggaguucgcugccuaccuggagccauucaaggagaagggcgagguuagacggccuacccucuccuggccucgcgagaucccucucguuaagggaggcaagcccgacgucguccagauuguccgcaacuacaacgccuaccuucgggccagcgacgaucugccuaagauguucaucgaguccgacccuggguucuuuuccaacgcuauugucgagggagcuaagaaguucccuaacaccgaguucgugaaggugaagggccuccacuucagccaggaggacgcuccagaugaaauggguaaguacaucaagagcuucg

SEQ ID NO: 6 - DNA, 42 bp, Artificial Sequence
  R primer
gaaggatccttacaggtcctcctctgagatcagcttctgctc

SEQ ID NO: 7 - DNA, 33 bp, Artificial Sequence
  F primer
gcagaattcaccatggcttccaaggtgtacgac

SEQ ID NO: 8 - DNA, 33 bp, Artificial Sequence
  F primer
gacgctagcaccatggcttccaaggtgtacgac

SEQ ID NO: 9 - DNA, 21 bp, Artificial Sequence
  R primer
cagctcgaactaagcggtgag

SEQ ID NO: 10 - DNA, 42 bp, Artificial Sequence
  R primer
gaactcgagttacaggtcctcctctgagatcagcttctgctc

SEQ ID NO: 11 - DNA, 21 bp, Artificial Sequence
  F primer
ctcaccgcttagttcgagctg

SEQ ID NO: 12 - DNA, 39 bp, Artificial Sequence
  F rpimer
ctaatacgactcactatagggctggactccttcatcaac

SEQ ID NO: 13 - DNA, 19 bp, Artificial Sequence
  R primer
ccagtcgtggcccacaaag

SEQ ID NO: 14 - DNA, 936 bp, Artificial Sequence
  Target Rluc mt
atggcttccaaggtgtacgaccccgagcaacgcaaacgcatgatcactgggcctcagtggtgggctcgctgcaagcaaatgaacgtgctggactccttcatcaactactatgattccgagaggcacgccgagaacgccgtgatttttctgcatggtaacgctgcctccagctacctgtggaggcacgtcgtgcctcacatcgagcccgtggctagatgcatcatccctgatctgatcggaatgggtaagtccggcaagagcgggaatggctcatatcgcctcctggatcactacaagtacctcaccgcttagttcgagctgctgaaccttccaaagaaaatcatctttgtgggccacgactggggggcttgtctggcctttcactactcctacgagcaccaagacaagatcaaggccatcgtccatgctgagagtgtcgtggacgtgatcgagtcctgggacgagtggcctgacatcgaggaggatatcgccctgatcaagagcgaagagggcgagaaaatggtgcttgagaataacttcttcgtcgagaccatgctcccaagcaagatcatgcggaaactggagcctgaggagttcgctgcctacctggagccattcaaggagaagggcgaggttagacggcctaccctctcctggcctcgcgagatccctctcgttaagggaggcaagcccgacgtcgtccagattgtccgcaactacaacgcctaccttcgggccagcgacgatctgcctaagatgttcatcgagtccgaccctgggttcttttccaacgctattgtcgagggagctaagaagttccctaacaccgagttcgtgaaggtgaagggcctccacttcagccaggaggacgctccagatgaaatgggtaagtacatcaagagcttcgtggagcgcgtgctgaagaacgagcagtaa

SEQ ID NO: 15 - RNA, 279 nt, Artificial Sequence
  Target s
gggcuggacuccuucaucaacuacuaugauuccgagaggcacgccgagaacgccgugauuuuucugcaugguaacgcugccuccagcuaccuguggaggcacgucgugccucacaucgagcccguggcuagaugcaucaucccugaucugaucggaauggguaaguccggcaagagcgggaauggcucauaucgccuccuggaucacuacaaguaccucaccgcuuaguucgagcugcugaaccuuccaaagaaaaucaucuuugugggccacgacugg

SEQ ID NO: 16 - DNA, 37 bp, Artificial Sequence
  primer
ggccacgcgtcgactagtacttttttttttttttttt

SEQ ID NO: 17 - DNA, 42 bp, Artificial Sequence
  primer
ctaatacgactcactatagggaccatggcttccaaggtgtac

SEQ ID NO: 18 - DNA, 20 bp, Artificial Sequence
  primer
ggccacgcgtcgactagtac

SEQ ID NO: 19 - DNA, 22 bp, Artificial Sequence
  primer
ttactgctcgttcttcagcacg

SEQ ID NO: 20 - DNA, 19 bp, Artificial Sequence
  primer
gctggactccttcatcaac

SEQ ID NO: 21 - DNA, 27 bp, Artificial Sequence
  primer
ctcaagatcatcagcaatgcctcctgc

SEQ ID NO: 22 - DNA, 36 bp, Artificial Sequence
  primer
gagcacagggtactttattgatggtacatgacaagg

SEQ ID NO: 23 - DNA, 22 bp, Artificial Sequence
  primer
gtatgacaacgaatttggctac

SEQ ID NO: 24 - RNA, 24 nt, Artificial Sequence
  gRNA
cagaguccccgaagccaucaaggg

SEQ ID NO: 25 - RNA, 24 nt, Artificial Sequence
  gRNA
gcccuuuuccgcaucacucgaacc

SEQ ID NO: 26 - RNA, 24 nt, Artificial Sequence
  gRNA
ugauccuuccacccagugguacaa

SEQ ID NO: 27 - RNA, 24 nt, Artificial Sequence
  gRNA
cuccacuggcacguauaucucugc

SEQ ID NO: 28 - RNA, 24 nt, Artificial Sequence
  gRNA
uaaaaucuccgucucugauguaca

SEQ ID NO: 29 - DNA, 57 bp, Artificial Sequence
  F primer
aattccgtgctgcagccccttgatggcttcagggaactctgccacaggtgagcctga

SEQ ID NO: 30 - DNA, 57 bp, Artificial Sequence
  R Primer
agcttcaggctcacctgtggcagagttccctgaagccatcaaggggctgcagcacgg

SEQ ID NO: 31 - DNA, 21 bp, Artificial Sequence
  F primer
caactgttgggaagggcgatc

SEQ ID NO: 32 - DNA, 23 bp, Artificial Sequence
  R primer
cgacaggtttcccgactggaaag

SEQ ID NO: 33 - DNA, 41 bp, Artificial Sequence
  F primer
ctaatacgactcactatagggcctcttcgctattacgccag

SEQ ID NO: 34 - DNA, 24 bp, Artificial Sequence
  R primer
ggaaacagctatgaccatgattac

SEQ ID NO: 35 - DNA, 21 bp, Artificial Sequence
  primer
ctaatacgactcactataggg

SEQ ID NO: 36 - DNA, 57 bp, Artificial Sequence
  F primer
aattcagcaaagagatggttcgagtgatgcagaagaagggcattgagcatcatccca

SEQ ID NO: 37 - DNA, 57 bp, Artificial Sequence
  R primer
agcttgggatgatgctcaatgcccttcttctgcatcactcgaaccatctctttgctg

SEQ ID NO: 38 - DNA, 57 bp, Artificial Sequence
  F primer
aattccacagctgcaattgtaccactgggtagaaaggatcattctgcacagagcaca

SEQ ID NO: 39 - DNA, 57 bp, Artificial Sequence
  R primer
agcttgtgctctgtgcagaatgatcctttctacccagtggtacaattgcagctgtgg

SEQ ID NO: 40 - DNA, 57 bp, Artificial Sequence
  F primer
aattccctggggaagagcagagatatacgtaccaggtggagcacccaggcctggata

SEQ ID NO: 41 - DNA, 57 bp, Artificial Sequence
  R primer
agcttatccaggcctgggtgctccacctggtacgtatatctctgctcttccccaggg

SEQ ID NO: 42 - DNA, 57 bp, Artificial Sequence
  F primer
aattctgacgcctcgttgtacatcagagacagagcattttacaccttgaagacgtaa

SEQ ID NO: 43 - DNA, 57 bp, Artificial Sequence
  R primer
agctttacgtcttcaaggtgtaaaatgctctgtctctgatgtacaacgaggcgtcag

SEQ ID NO: 44 - DNA, 32 bp, Artificial Sequence
  F primer
gtactcgaggggcctcttcgctattacgccag

SEQ ID NO: 45 - DNA, 28 bp, Artificial Sequence
  R primer
gatggtaccggaaacagctatgaccatg

SEQ ID NO: 46 - DNA, 19 bp, Artificial Sequence
  F primer
tggcaccaaaatcaacggg

SEQ ID NO: 47 - DNA, 22 bp, Artificial Sequence
  R primer
gctattgtcttcccaatcctcc

SEQ ID NO: 48 - DNA, 20 bp, Artificial Sequence
  primer
ggccacgcgtcgactagtac

SEQ ID NO: 49 - RNA, 24 nt, Artificial Sequence
  gRNA for Factor V
cuguauccucgccuguccagggau

SEQ ID NO: 50 - RNA, 24 nt, Artificial Sequence
  gRNA for PAH.1
guggaaacucggaaggccaggcca

SEQ ID NO: 51 - RNA, 24 nt, Artificial Sequence
  gRNA for ASS1
uugaugacccgguggcaucaguug

SEQ ID NO: 52 - RNA, 24 nt, Artificial Sequence
  gRNA for GFAP
auacuggugcggaucucuuucagg

SEQ ID NO: 53 - RNA, 24 nt, Artificial Sequence
  gRNA for CBS
ggcgccggucgaagcccuucuccc

SEQ ID NO: 54 - RNA, 24 nt, Artificial Sequence
  gRNA for GRIA2
gcauccugccgcauaaaggcaccc

SEQ ID NO: 55 - RNA, 24 nt, Artificial Sequence
  gRNA for SLCO2A1
gggucauuacguuuaaugaaaucc

SEQ ID NO: 56 - RNA, 24 nt, Artificial Sequence
  gRNA for RL_A287_GC
cuuguaugacccaggaggcgauau

SEQ ID NO: 57 - RNA, 24 nt, Artificial Sequence
  gRNA for RL_A287_GG
cuuguaugacgcaggaggcgauau

SEQ ID NO: 58 - RNA, 24 nt, Artificial Sequence
  gRNA for RL_A287_U
cuuguaugacucaggaggcgauau

SEQ ID NO: 59 - RNA, 24 nt, Artificial Sequence
  rRNA for RL_A287_A
cuuguaugacacaggaggcgauau

SEQ ID NO: 60 - RNA, 24 nt, Artificial Sequence
  gRNA for  PAH.2
cuguagccccaagugaaaaguuau

SEQ ID NO: 61 - RNA, 24 nt, Artificial Sequence
  gRNA for PANK2
aagaaauuccaacaaauaccaccu

SEQ ID NO: 62 - RNA, 24 nt, Artificial Sequence
  gRNA for NPHS2
auguccagucggaauauaauuacu

SEQ ID NO: 63 - RNA, 24 nt, Artificial Sequence
  gRNA for A1AT
gucccuucucgucgauggucagca

SEQ ID NO: 64 - DNA, 57 bp, Artificial Sequence
  F primer
aattctctcccctcctcacagttgccatgtagaccccttgaagaggggaggggccta

SEQ ID NO: 65 - DNA, 57 bp, Artificial Sequence
  RV primer
agcttaggcccctcccctcttcaaggggtctacatggcaactgtgaggaggggagag

SEQ ID NO: 66 - DNA, 30 bp, Artificial Sequence
  primer
gcagaattcgggctggactccttcatcaac

SEQ ID NO: 67 - DNA, 26 bp, Artificial Sequence
  primer
cttgtagtgattcaggaggcgatatg

SEQ ID NO: 68 - DNA, 26 bp, Artificial Sequence
  primer
catatcgcctcctgaatcactacaag

SEQ ID NO: 69 - DNA, 28 bp, Artificial Sequence
  primer
cgtaagcttccagtcgtggcccacaaag

SEQ ID NO: 70 - DNA, 39 bp, Artificial Sequence; identical to SEQ ID NO: 12
  primer

SEQ ID NO: 71 - DNA, 19 bp, Artificial Sequence
  primer
ccagtcgtggcccacaaag

SEQ ID NO: 72 - DNA, 297 bp, Artificial Sequence
  Rluc_sRNA_G286A_Eco/Hind
gcaggatccgggctggactccttcatcaactactatgattccgagaggcacgccgagaacgccgtgatttttctgcatggtaacgctgcctccagctacctgtggaggcacgtcgtgcctcacatcgagcccgtggctagatgcatcatccctgatctgatcggaatgggtaagtccggcaagagcgggaatggctcatatcgcctcctgaatcactacaagtacctcaccgcttagttcgagctgctgaaccttccaaagaaaatcatctttgtgggccacgactggaagcttacg

SEQ ID NO: 73 - RNA, 279 nt, Artificial Sequence
  Rluc_sRNA_G286A
gggcuggacuccuucaucaacuacuaugauuccgagaggcacgccgagaacgccgugauuuuucugcaugguaacgcugccuccagcuaccuguggaggcacgucgugccucacaucgagcccguggcuagaugcaucaucccugaucugaucggaauggguaaguccggcaagagcgggaauggcucauaucgccuccugaaucacuacaaguaccucaccgcuuaguucgagcugcugaaccuuccaaagaaaaucaucuuugugggccacgacugg

SEQ ID NO: 74 - DNA, 30 bp, Artificial Sequence
  primer
gcaggatccgggctggactccttcatcaac

SEQ ID NO: 75 - DNA, 28 bp, Artificial Sequence
  primer
cgtaagcttccagtcgtggcccacaaag

SEQ ID NO: 76 - DNA, 19 bp, Artificial Sequence
  primer
tggcaccaaaatcaacggg

SEQ ID NO: 77 - DNA, 22 bp, Artificial Sequence
  primer
gctattgtcttcccaatcctcc

SEQ ID NO: 78 - DNA, 19 bp, Artificial Sequence
  primer
gctggactccttcatcaac

SEQ ID NO: 79 - DNA, 19 bp, Artificial Sequence
  primer
ccagtcgtggcccacaaag

SEQ ID NO: 80 - DNA, 29 bp, Artificial Sequence
  primer
cgatctagaatgccgtcttctgtctcgtg

SEQ ID NO: 81 - DNA, 31 bp, Artificial Sequence
  primer
gcaaagcttttatttttgggtgggattcacc

SEQ ID NO: 82 - DNA, 21 bp, Artificial Sequence
  primer
caactgttgggaagggcgatc

SEQ ID NO: 83 - DNA, 23 bp, Artificial Sequence
  primer
cgacaggtttcccgactggaaag

SEQ ID NO: 84 - DNA, 21 bp, Artificial Sequence
  primer
gtccctttcttgtcgatggtc

SEQ ID NO: 85 - DNA, 21 bp, Artificial Sequence
  primer
gaccatcgacaagaaagggac

SEQ ID NO: 86 - DNA, 19 bp, Artificial Sequence
  primer
tggcaccaaaatcaacggg

SEQ ID NO: 87 - DNA, 22 bp, Artificial Sequence
  primer
gctattgtcttcccaatcctcc

SEQ ID NO: 88 - DNA, 1275 bp, Artificial Sequence
  SERPINA1_CDS
cgatctagaatgccgtcttctgtctcgtggggcatcctcctgctggcaggcctgtgctgcctggtccctgtctccctggctgaggatccccagggagatgctgcccagaagacagatacatcccaccatgatcaggatcacccaaccttcaacaagatcacccccaacctggctgagttcgccttcagcctataccgccagctggcacaccagtccaacagcaccaatatcttcttctccccagtgagcatcgctacagcctttgcaatgctctccctggggaccaaggctgacactcacgatgaaatcctggagggcctgaatttcaacctcacggagattccggaggctcagatccatgaaggcttccaggaactcctccgtaccctcaaccagccagacagccagctccagctgaccaccggcaatggcctgttcctcagcgagggcctgaagctagtggataagtttttggaggatgttaaaaagttgtaccactcagaagccttcactgtcaacttcggggacaccgaagaggccaagaaacagatcaacgattacgtggagaagggtactcaagggaaaattgtggatttggtcaaggagcttgacagagacacagtttttgctctggtgaattacatcttctttaaaggcaaatgggagagaccctttgaagtcaaggacaccgaggaagaggacttccacgtggaccaggtgaccaccgtgaaggtgcctatgatgaagcgtttaggcatgtttaacatccagcactgtaagaagctgtccagctgggtgctgctgatgaaatacctgggcaatgccaccgccatcttcttcctgcctgatgaggggaaactacagcacctggaaaatgaactcacccacgatatcatcaccaagttcctggaaaatgaagacagaaggtctgccagcttacatttacccaaactgtccattactggaacctatgatctgaagagcgtcctgggtcaactgggcatcactaaggtcttcagcaatggggctgacctctccggggtcacagaggaggcacccctgaagctctccaaggccgtgcataaggctgtgctgaccatcgacgagaaagggactgaagctgctggggccatgtttttagaggccatacccatgtctatcccccccgaggtcaagttcaacaaaccctttgtcttcttaatgattgaacaaaataccaagtctcccctcttcatgggaaaagtggtgaatcccacccaaaaataaaagctttgc

SEQ ID NO: 89 - DNA, 1275 bp, Artificial Sequence
  SERPINA1_G1096A
cgatctagaatgccgtcttctgtctcgtggggcatcctcctgctggcaggcctgtgctgcctggtccctgtctccctggctgaggatccccagggagatgctgcccagaagacagatacatcccaccatgatcaggatcacccaaccttcaacaagatcacccccaacctggctgagttcgccttcagcctataccgccagctggcacaccagtccaacagcaccaatatcttcttctccccagtgagcatcgctacagcctttgcaatgctctccctggggaccaaggctgacactcacgatgaaatcctggagggcctgaatttcaacctcacggagattccggaggctcagatccatgaaggcttccaggaactcctccgtaccctcaaccagccagacagccagctccagctgaccaccggcaatggcctgttcctcagcgagggcctgaagctagtggataagtttttggaggatgttaaaaagttgtaccactcagaagccttcactgtcaacttcggggacaccgaagaggccaagaaacagatcaacgattacgtggagaagggtactcaagggaaaattgtggatttggtcaaggagcttgacagagacacagtttttgctctggtgaattacatcttctttaaaggcaaatgggagagaccctttgaagtcaaggacaccgaggaagaggacttccacgtggaccaggtgaccaccgtgaaggtgcctatgatgaagcgtttaggcatgtttaacatccagcactgtaagaagctgtccagctgggtgctgctgatgaaatacctgggcaatgccaccgccatcttcttcctgcctgatgaggggaaactacagcacctggaaaatgaactcacccacgatatcatcaccaagttcctggaaaatgaagacagaaggtctgccagcttacatttacccaaactgtccattactggaacctatgatctgaagagcgtcctgggtcaactgggcatcactaaggtcttcagcaatggggctgacctctccggggtcacagaggaggcacccctgaagctctccaaggccgtgcataaggctgtgctgaccatcgacaagaaagggactgaagctgctggggccatgtttttagaggccatacccatgtctatcccccccgaggtcaagttcaacaaaccctttgtcttcttaatgattgaacaaaataccaagtctcccctcttcatgggaaaagtggtgaatcccacccaaaaataaaagctttgc

SEQ ID NO: 90 - DNA, 23 bp, Artificial Sequence
  primer
ggcatgtttaacatccagcactg

SEQ ID NO: 91 - DNA, 31 bp, Artificial Sequence; identical to SEQ ID NO: 81
  primer

SEQ ID NO: 92 - DNA, 21 bp, Artificial Sequence
  primer
ccatcttcttcctgcctgatg

SEQ ID NO: 93 - DNA, 20 bp, Artificial Sequence
  primer
catgaagaggggagacttgg

SEQ ID NO: 94 - DNA, 23 bp, Artificial Sequence
  primer
gaactcacccacgatatcatcac

SEQ ID NO: 95 - DNA, 57 bp, Artificial Sequence
  primer
aattctgtaagagcagatccctggacaggcaaggaatacaggtattttgtccttgaa

SEQ ID NO: 96 - DNA, 57 bp, Artificial Sequence
  primer
agctttcaaggacaaaatacctgtattccttgcctgtccagggatctgctcttacag

SEQ ID NO: 97 - DNA, 57 bp, Artificial Sequence
  primer
aattccgagatcctccgggagaagggcttcaaccaggcgcccgtggtggatgaggca

SEQ ID NO: 98 - DNA, 57 bp, Artificial Sequence
  primer
agcttgcctcatccaccacgggcgcctggttgaagcccttctcccggaggatctcgg

SEQ ID NO: 99 - DNA, 57 bp, Artificial Sequence
  primer
aattctaacagtgataataacttttcacttagggcctacagtactgcttatcagaga

SEQ ID NO: 100 - DNA, 57 bp, Artificial Sequence
  primer
agcttctctgataagcagtactgtaggccctaagtgaaaagttattatcactgttag

SEQ ID NO: 101 - DNA, 57 bp, Artificial Sequence
  primer
aattctgattatgagccaactgatgccaccaggttcatcaacatcaattccctcaga

SEQ ID NO: 102 - DNA, 57 bp, Artificial Sequence
  primer
agcttctgagggaattgatgttgatgaacctggtggcatcagttggctcataatcag

SEQ ID NO: 103 - DNA, 57 bp, Artificial Sequence
  primer
aattctggttttccttgggtgcctttatgcagcaaggatgcgatatttcgccaagaa

SEQ ID NO: 104 - DNA, 57 bp, Artificial Sequence
  primer
agctttcttggcgaaatatcgcatccttgctgcataaaggcacccaaggaaaaccag

SEQ ID NO: 105 - DNA, 57 bp, Artificial Sequence
  primer
aattcggctccctggtggatttcattaaacataactgaccctacagccctgggtgga

SEQ ID NO: 106 - DNA, 57 bp, Artificial Sequence
  primer
agcttccacccagggctgtagggtcagttatgtttaatgaaatccaccagggagccg

SEQ ID NO: 107 - DNA, 57 bp, Artificial Sequence
  primer
aattcctcaccgcagccctgaaagagatccacacgcagtatgaggcaatggcgtcca

SEQ ID NO: 108 - DNA, 57 bp, Artificial Sequence
  primer
agcttggacgccattgcctcatactgcgtgtggatctctttcagggctgcggtgagg

SEQ ID NO: 109 - DNA, 57 bp, Artificial Sequence
  primer
aattcaaacattaaccaggtggtatttgttagaaatttcttgagaattaatacgata

SEQ ID NO: 110 - DNA, 57 bp, Artificial Sequence
  primer
agcttatcgtattaattctcaagaaatttctaacaaataccacctggttaatgtttg

SEQ ID NO: 111 - DNA, 57 bp, Artificial Sequence
  primer
aattcgagtatgaaagagtaattatattccaactgggacatctgcttcctggaagaa

SEQ ID NO: 112 - DNA, 57 bp, Artificial Sequence
  primer
agctttcttccaggaagcagatgtcccagttggaatataattactctttcatactcg